European Patent Application EP 4 610 267 A1, published September 3, 2025. Title: Cyclic dinucleotides and conjugates thereof with antibodies. Applicant: Ustav organicke chemie a biochemie AV CR, v. v. i. Application EP. The sequence listing filed with the application follows.

SEQUENCE LISTING (38 sequences)

SEQ ID NO: 1 - DNA, 1350 bp, synthetic construct
  source 1..1350: mol_type = other DNA
gaagtgcagctggtggaaagcggcggcggcctggtgcagccgggcggcagcctgcgcctgagctgcgcggcgagcggctttaacattaaagatacctatattcattgggtgcgccaggcgccgggcaaaggcctggaatgggtggcgcgcatttatccgaccaacggctatacccgctatgcggatagcgtgaaaggccgctttaccattagcgcggataccagcaaaaacaccgcgtatctgcagatgaacagcctgcgcgcggaagataccgcggtgtattattgcagccgctggggcggcgatggcttttatgcgatggattattggggccagggcaccctggtgaccgtgagcagcgcgagcaccaaaggcccgagcgtgtttccgctggcgccgagcagcaaaagcaccagcggcggcaccgcggcgctgggctgcctggtcaaggactattttccgtgtccggtgaccgtgagctggaacagcggcgcgctgaccagcggcgtgcatacctttccggcggtgctgcagagcagcggcctgtatagcctgagcagcgtggtgaccgtgccgagcagcagcctgggcacccagacctatatttgcaacgtgaaccataaaccgagcaacaccaaagtggataaaaaagtggaaccgaaaagctgcgataaaacccatacctgcccgccgtgcccggcgccggaactgctgggcggcccgagcgtgtttctgtttccgccgaaaccgaaagataccctgatgattagccgcaccccggaagtgacctgcgtggtggtggatgtgagccatgaagatccggaagtgaaatttaactggtatgtggatggcgtggaagtgcataacgcgaaaaccaaaccgcgcgaagaacagtataacagcacctatcgcgtggtgagcgtgctgaccgtgctgcatcaggattggctgaacggcaaagaatataaatgcaaagtgagcaacaaagcgctgccggcgccgattgaaaaaaccattagcaaagcgaaaggccagccgcgcgaaccgcaggtgtataccctgccgccgagccgcgaagaaatgaccaaaaaccaggtgagcctgacctgcctggtgaaaggcttttatccgtgcgatattgcggtggaatgggaaagcaacggccagccggaaaacaactataaaaccaccccgccggtgctggatagcgatggcagcttttttctgtatagcaaactgaccgtggataaaagccgctggcagcagggcaacgtgtttagctgcagcgtgatgcatgaagcgctgcataaccattatacccagaaaagcctgagcctgagcccgggcaaa

SEQ ID NO: 2 - DNA, 723 bp, synthetic construct
  source 1..723: mol_type = other DNA
gcttccaccatgtctgtgcctacacaggtgctgggactgctgctgctgtggctgacagatgccagatgcgacatccagatgacacagagccctagcagcctgtctgccagcgtgggagacagagtgaccatcacctgtagagccagccaggacgtgaacacagccgtggcttggtatcagcagaagcctggcaaggcccctaagctgctgatctacagcgccagctttctgtacagcggcgtgcccagcagattcagcggctctagaagcggcaccgacttcaccctgaccataagcagtctgcagcccgaggacttcgccacctactactgtcagcagcactacaccacacctccaacctttggccagggcaccaaggtggaaatcaagcggacagtggccgctcctagcgtgttcatctttccacctagcgacgagcagctgaagtctggcacagcctctgtcgtgtgcctgctgaacaacttctaccccagagaagccaaggtgcagtggaaggtggacaacgccctgcagagcggcaatagccaagagagcgtgaccgagcaggacagcaaggactctacctacagcctgagcagcaccctgacactgagcaaggccgactacgagaagcacaaagtgtacgcctgcgaagtgacccaccagggcctttctagccctgtgaccaagagcttcaaccggggcgagtgctgatagctcgag

SEQ ID NO: 3 - DNA, 1350 bp, synthetic construct
  source 1..1350: mol_type = other DNA
gaagtgcagctggtggaaagcggcggcggcctggtgcagccgggcggcagcctgcgcctgagctgcgcggcgagcggctttaacattaaagatacctatattcattgggtgcgccaggcgccgggcaaaggcctggaatgggtggcgcgcatttatccgaccaacggctatacccgctatgcggatagcgtgaaaggccgctttaccattagcgcggataccagcaaaaacaccgcgtatctgcagatgaacagcctgcgcgcggaagataccgcggtgtattattgcagccgctggggcggcgatggcttttatgcgatggattattggggccagggcaccctggtgaccgtgagcagcgcgagcaccaaaggcccgagcgtgtttccgctggcgccgagcagcaaaagcaccagcggcggcaccgcggcgctgggctgcctggtcaaggactattttccggagccggtgaccgtgagctggaacagcggcgcgctgaccagcggcgtgcatacctttccggcggtgctgcagagcagcggcctgtatagcctgagcagcgtggtgaccgtgccgagcagcagcctgggcacccagacctatatttgcaacgtgaaccataaaccgagcaacaccaaagtggataaaaaagtggaaccgaaaagctgcgataaaacccatacctgcccgccgtgcccggcgccggaactgctgggcggcccgagcgtgtttctgtttccgccgaaaccgaaagataccctgatgattagccgcaccccggaagtgacctgcgtggtggtggatgtgagccatgaagatccggaagtgaaatttaactggtatgtggatggcgtggaagtgcataacgcgaaaaccaaaccgcgcgaagaacagtataacagcacctatcgcgtggtgagcgtgctgaccgtgctgcatcaggattggctgaacggcaaagaatataaatgcaaagtgagcaacaaagcgctgccggcgccgattgaaaaaaccattagcaaagcgaaaggccagccgcgcgaaccgcaggtgtataccctgccgccgagccgcgaagaaatgaccaaaaaccaggtgagcctgacctgcctggtgaaaggcttttatccgagcgatattgcggtggaatgggaaagcaacggccagccggaaaacaactataaaaccaccccgccggtgctggatagcgatggcagcttttttctgtatagcaaactgaccgtggataaaagccgctggcagcagggcaacgtgtttagctgcagcgtgatgcatgaagcgctgcataaccattatacccagaaaagcctgagcctgagcccgggcaaa

SEQ ID NO: 4 - DNA, 723 bp, synthetic construct; identical to SEQ ID NO: 2
  source 1..723: mol_type = other DNA

SEQ ID NO: 5 - DNA, 1350 bp, synthetic construct
  source 1..1350: mol_type = other DNA
gaagtgcagctggtggaaagcggcggcggcctggtgcagccgggcggcagcctgcgcctgagctgcgcggcgagcggctttaacattaaagatacctatattcattgggtgcgccaggcgccgggcaaaggcctggaatgggtggcgcgcatttatccgaccaacggctatacccgctatgcggatagcgtgaaaggccgctttaccattagcgcggataccagcaaaaacaccgcgtatctgcagatgaacagcctgcgcgcggaagataccgcggtgtattattgcagccgctggggcggcgatggcttttatgcgatggattattggggccagggcaccctggtgaccgtgagcagcgcgagcaccaaaggcccgagcgtgtttccgctggcgccgagcagcaaaagcaccagcggcggcaccgcggcgctgggctgcctggtcaaggactattttccggagccggtgaccgtgagctggaacagcggcgcgctgaccagcggcgtgcatacctttccggcggtgctgcagagcagcggcctgtatagcctgagcagcgtggtgaccgtgccgagcagcagcctgggcacccagacctatatttgcaacgtgaaccataaaccgagcaacaccaaagtggataaaaaagtggaaccgaaaagctgcgataaaacccatacctgcccgccgtgcccggcgccggaactgctgggcggcccgagcgtgtttctgtttccgccgaaaccgaaagataccctgatgattagccgcaccccggaagtgacctgcgtggtggtggatgtgagccatgaagatccggaagtgaaatttaactggtatgtggatggcgtggaagtgcataacgcgaaaaccaaaccgcgcgaagaacagtataacagcacctatcgcgtggtgagcgtgctgaccgtgctgcatcaggattggctgaacggcaaagaatataaatgcaaagtgagcaacaaagcgctgccggcgccgattgaaaaaaccattagcaaagcgaaaggccagccgcgcgaaccgcaggtgtataccctgccgccgagccgcgaagaaatgaccaaaaaccaggtgagcctgacctgcctggtgaaaggcttttatccgtgcgatattgcggtggaatgggaaagcaacggccagccggaaaacaactataaaaccaccccgccggtgctggatagcgatggcagcttttttctgtatagcaaactgaccgtggataaaagccgctggcagcagggcaacgtgtttagctgcagcgtgatgcatgaagcgctgcataaccattatacccagaaaagcctgagcctgagcccgggcaaa

SEQ ID NO: 6 - DNA, 725 bp, synthetic construct
  source 1..725: mol_type = other DNA
aagcttccaccatgtctgtgcctacacaggtgctgggactgctgctgctgtggctgacagatgccagatgcgacatccagatgacacagagccctagcagcctgtctgccagcgtgggagacagagtgaccatcacctgtagagccagccaggacgtgaacacagccgtggcttggtatcagcagaagcctggcaaggcccctaagctgctgatctacagcgccagctttctgtacagcggcgtgcccagcagattcagcggctctagaagcggcaccgacttcaccctgaccataagcagtctgcagcccgaggacttcgccacctactactgtcagcagcactacaccacacctccaacctttggccagggcaccaaggtggaaatcaagcggacatgcgccgctcctagcgtgttcatctttccacctagcgacgagcagctgaagtctggcacagcctctgtcgtgtgcctgctgaacaacttctaccccagagaagccaaggtgcagtggaaggtggacaacgccctgcagagcggcaatagccaagagagcgtgaccgagcaggacagcaaggactctacctacagcctgagcagcaccctgacactgagcaaggccgactacgagaagcacaaagtgtacgcctgcgaagtgacccaccagggcctttctagccctgtgaccaagagcttcaaccggggcgagtgctgatagctcgag

SEQ ID NO: 7 - DNA, 1352 bp, synthetic construct
  source 1..1352: mol_type = other DNA
caggttcagctgcagcagtctggcagcgagctgaagaaacctggcgcctctgtgaaggtgtcctgcaaggccagcggctacacctttaccaactacggcatgaactgggtcaagcaggcccctggacagggcctgaaatggatgggctggatcaacacctacaccggcgagcccacctacacagacgacttcaagggcagattcgccttcagcctggacacctctgtgtccacagcctacctgcagatcagcagcctgaaggccgatgataccgccgtgtacttctgtgccagaggcggctttggcagcagctactggtacttcgatgtgtggggccagggcagcctggtcacagttagctctgcctctacaaagggccccagcgtgttccctctggctcctagcagcaagtctacaagcggaggaacagccgctctgggctgcctcgtgaaggattactttcccgagcctgtgaccgtgtcctggaattctggcgctctgacaagcggcgtgcacacctttccagctgtgctgcaaagcagcggcctgtactctctgagcagcgtcgtgacagtgcctagcagctctctgggcacccagacctacatctgcaatgtgaaccacaagcctagcaacaccaaggtggacaagagagtggaacccaagagctgcgacaagacccacacctgtcctccatgtcctgctccagaactgctcggcggaccttccgtgtttctgttccctccaaagcctaaggacaccctgatgatcagcagaacccctgaagtgacctgcgtggtggtggatgtgtcccacgaggatcccgaagtgaagttcaattggtacgtggacggcgtggaagtgcacaacgccaagaccaagcctagagaggaacagtacaacagcacctacagagtggtgtccgtgctgaccgtgctgcaccaggattggctgaacggcaaagagtacaagtgcaaggtgtccaacaaggctctgcccgctcctatcgagaaaaccatcagcaaggccaagggccagcctagggaaccccaggtttacacactgcctccaagccgggaagagatgaccaagaaccaggtgtccctgacctgcctggtcaagggcttctacccttccgatatcgccgtggaatgggagagcaatggccagcctgagaacaactacaagacaacccctcctgtgctggacagcgacggctcattcttcctgtacagcaagctgacagtggacaagtccagatggcagcagggcaacgtgttctcctgctccgtgatgcacgaggccctgcacaaccactacacccagaagtccctgagcctgtctcctggcaa

SEQ ID NO: 8 - DNA, 642 bp, synthetic construct
  source 1..642: mol_type = other DNA
gacatccagctgacacagagccctagcagcctgtctgcctctgtgggcgacagagtgtccatcacatgcaaggccagccaggacgtgtcaattgccgtggcctggtatcagcagaagcctggcaaagcccctaagctgctgatctacagcgccagctacagatacaccggcgtgcccgatagattttccggctctggcagcggcaccgacttcaccctgaccatatctagcctgcagcctgaggacttcgccgtgtactactgccagcagcactacatcacccctctgacctttggagccggcaccaaggtggaaatcaagcggacagtggccgctcctagcgtgttcatctttccacctagcgacgagcagctgaagtctggcacagcctctgtcgtgtgcctgctgaacaacttctaccccagagaagccaaggtgcagtggaaggtggacaacgccctgcagagcggcaatagccaagagagcgtgaccgagcaggacagcaaggactctacctactctctgagcagcaccctgacactgagcaaggccgactacgagaagcacaaagtgtacgcctgcgaagtgacccaccagggcctttctagccctgtgaccaagagcttcaaccggggcgagtgc

SEQ ID NO: 9 - DNA, 1353 bp, synthetic construct
  source 1..1353: mol_type = other DNA
caggttcagctgcagcagtctggcagcgagctgaagaaacctggcgcctctgtgaaggtgtcctgcaaggccagcggctacacctttaccaactacggcatgaactgggtcaagcaggcccctggacagggcctgaaatggatgggctggatcaacacctacaccggcgagcccacctacacagacgacttcaagggcagattcgccttcagcctggacacctctgtgtccacagcctacctgcagatcagcagcctgaaggccgatgataccgccgtgtacttctgtgccagaggcggctttggcagcagctactggtacttcgatgtgtggggccagggcagcctggtcacagttagctctgcctctacaaagggccccagcgttttcccactggctcctagcagcaagagcacaagcggaggaacagctgctctgggctgcctggtcaaggactatttccccgagcctgtgaccgtgtcctggaactctggcgctctgacttctggcgtgcacacctttccagccgtgctgcaaagcagcggcctgtactctctgagcagcgtcgtgacagtgccaagctctagcctgggcacccagacctacatctgcaatgtgaaccacaagcctagcaacaccaaggtggacaagaaggtggaacccaagagctgcgacaagacccacacctgtcctccatgtcctgctccagaactgctcggcggaccttccgtgtttctgttccctccaaagcctaaggacaccctgatgatcagcagaacccctgaagtgacctgcgtggtggtggatgtgtcccacgaggatcccgaagtgaagttcaattggtacgtggacggcgtcgaggtgcacaacgccaagacaaagcccagagaggaacagtacaacagcacctacagagtggtgtccgtgctgacagtgctgcaccaggattggctgaacggcaaagagtacaagtgcaaggtgtccaacaaggccctgcctgctcctatcgagaaaaccatcagcaaggccaagggccagcctagagaaccccaggtgtacacactgcctccaagccgggaagagatgaccaagaaccaggtgtccctgacctgtctcgtgaagggcttctacccctgcgacattgccgtggaatgggagagcaatggacagcccgagaacaactacaagacaacccctcctgtgctggacagcgacggctcattcttcctgtacagcaagctgaccgtggacaagtccagatggcagcagggcaacgtgttcagctgcagcgtgatgcacgaggccctgcacaaccactacacccagaagtccctgtctctgagccccggcaag

SEQ ID NO: 10 - DNA, 642 bp, synthetic construct
  source 1..642: mol_type = other DNA
gacatccagctgacacagagccctagcagcctgtctgcctctgtgggcgacagagtgtccatcacatgcaaggccagccaggacgtgtcaattgccgtggcctggtatcagcagaagcctggcaaagcccctaagctgctgatctacagcgccagctacagatacaccggcgtgcccgatagattttccggctctggcagcggcaccgacttcaccctgaccatatctagcctgcagcctgaggacttcgccgtgtactactgccagcagcactacatcacccctctgacctttggagccggcaccaaggtggaaatcaagcggacatgtgctgcccctagcgtgttcatcttcccaccttccgacgagcagctgaagtctggcacagcctctgtcgtgtgcctgctgaacaacttctaccccagagaagccaaggtgcagtggaaggtggacaacgccctgcagagcggcaatagccaagagagcgtgaccgagcaggacagcaaggactctacctactctctgagcagcaccctgacactgagcaaggccgactacgagaagcacaaagtgtacgcctgcgaagtgacccaccagggcctttctagccctgtgaccaagagcttcaaccggggcgagtgc

SEQ ID NO: 11 - DNA, 1347 bp, synthetic construct
  source 1..1347: mol_type = other DNA
gaagtgcagctggttgaatctggtggcggagtggtgcagcctggcagatctctgagactgagctgtagcgccagcggcttcaccttttctggctacggcctgagctgggtccgacaggctcctggaaaaggcctggaatgggtcgccatgatcagcagcggcggcagctacacctactacgccgattctgtgaagggcagattcgccatcagccgggacaacgccaagaataccctgttcctgcagatggacagcctgcggcctgaagataccggcgtgtacttctgtgccagacacggcgacgaccctgcttggtttgcttattggggccagggcacccctgtgacagtgtctagcgcctctacaaagggccccagcgttttcccactggctcctagcagcaagagcacctctggtggaacagccgctctgggctgtctggtcaaggactacttcccctgtccagtgaccgtgtcctggaattctggcgccctgacatctggcgtgcacacctttccagctgtgctgcagtctagcggcctgtactctctgagcagcgtggtcacagtgccaagctctagcctgggcacccagacctacatctgcaatgtgaaccacaagcctagcaacaccaaggtggacaagaaggtggaacccaagagctgcgacaagacccacacctgtcctccatgtcctgctccagaactgctcggcggaccttccgtgtttctgttccctccaaagcctaaggacaccctgatgatctccagaacacccgaagtgacctgcgtggtggtggatgtgtctcacgaggaccctgaagtgaagttcaattggtacgtggacggcgtcgaggtgcacaatgccaagaccaagcctagagaggaacagtacaacagcacctacagagtggtgtccgtgctgaccgtgctgcaccaggattggctgaacggcaaagagtacaagtgcaaggtgtccaacaaggccctgcctgctcctatcgagaaaaccatcagcaaggccaagggccagcctagggaaccccaggtttacacactgcctccaagccgggaagagatgaccaagaaccaggtgtccctgacctgcctcgtgaagggcttctacccctgcgacattgccgtggaatgggagagcaatggccagcctgagaacaactacaagacaacccctcctgtgctggactccgacggctcattcttcctgtacagcaagctgacagtggacaagtccagatggcagcagggcaacgtgttcagctgcagcgtgatgcacgaggccctgcacaaccactacacccagaagtccctgagcctgtctcctggcaag

SEQ ID NO: 12 - DNA, 651 bp, synthetic construct
  source 1..651: mol_type = other DNA
gacatccagctgacacagagccctagcagcctgtctgcctctgtgggcgacagagtgaccatcacctgtagcgtgtccagcagcatcagcagcaacaacctgcactggtatcagcagaagcccggcaaggcccctaagccttggatctacggcacaagcaatctggccagcggcgtgccaagcagattttctggctctggcagcggcaccgactacaccttcaccatatctagcctgcagcctgaggatatcgccacctactactgccagcagtggtctagctacccctacatgtacaccttcggccagggcaccaaggtggaaatcaagagaacagtggccgctcctagcgtgttcatcttcccaccttccgacgagcagctgaagtctggcacagcctctgtcgtgtgcctgctgaacaacttctaccccagagaagccaaggtgcagtggaaggtggacaacgccctgcagagcggcaatagccaagagagcgtgaccgagcaggacagcaaggactctacctactctctgagcagcaccctgacactgagcaaggccgactacgagaagcacaaagtgtacgcctgcgaagtgacccaccagggcctttctagccctgtgaccaagagcttcaaccggggcgagtgc

SEQ ID NO: 13 - protein, 450 aa, synthetic construct
EVQLVESGGGLVQPGGSLRLSCAASGFNIKDTYIHWVRQAPGKGLEWVARIYPTNGYTRYADSVKGRFTISADTSKNTAYLQMNSLRAEDTAVYYCSRWGGDGFYAMDYWGQGTLVTVSSASTKGPSVFPLAPSSKSTSGGTAALGCLVKDYFPCPVTVSWNSGALTSGVHTFPAVLQSSGLYSLSSVVTVPSSSLGTQTYICNVNHKPSNTKVDKKVEPKSCDKTHTCPPCPAPELLGGPSVFLFPPKPKDTLMISRTPEVTCVVVDVSHEDPEVKFNWYVDGVEVHNAKTKPREEQYNSTYRVVSVLTVLHQDWLNGKEYKCKVSNKALPAPIEKTISKAKGQPREPQVYTLPPSREEMTKNQVSLTCLVKGFYPCDIAVEWESNGQPENNYKTTPPVLDSDGSFFLYSKLTVDKSRWQQGNVFSCSVMHEALHNHYTQKSLSLSPGK

SEQ ID NO: 14 - protein, 214 aa, synthetic construct
DIQMTQSPSSLSASVGDRVTITCRASQDVNTAVAWYQQKPGKAPKLLIYSASFLYSGVPSRFSGSRSGTDFTLTISSLQPEDFATYYCQQHYTTPPTFGQGTKVEIKRTVAAPSVFIFPPSDEQLKSGTASVVCLLNNFYPREAKVQWKVDNALQSGNSQESVTEQDSKDSTYSLSSTLTLSKADYEKHKVYACEVTHQGLSSPVTKSFNRGEC

SEQ ID NO: 15 - protein, 450 aa, synthetic construct
EVQLVESGGGLVQPGGSLRLSCAASGFNIKDTYIHWVRQAPGKGLEWVARIYPTNGYTRYADSVKGRFTISADTSKNTAYLQMNSLRAEDTAVYYCSRWGGDGFYAMDYWGQGTLVTVSSASTKGPSVFPLAPSSKSTSGGTAALGCLVKDYFPEPVTVSWNSGALTSGVHTFPAVLQSSGLYSLSSVVTVPSSSLGTQTYICNVNHKPSNTKVDKKVEPKSCDKTHTCPPCPAPELLGGPSVFLFPPKPKDTLMISRTPEVTCVVVDVSHEDPEVKFNWYVDGVEVHNAKTKPREEQYNSTYRVVSVLTVLHQDWLNGKEYKCKVSNKALPAPIEKTISKAKGQPREPQVYTLPPSREEMTKNQVSLTCLVKGFYPSDIAVEWESNGQPENNYKTTPPVLDSDGSFFLYSKLTVDKSRWQQGNVFSCSVMHEALHNHYTQKSLSLSPGK

SEQ ID NO: 16 - protein, 214 aa, synthetic construct; identical to SEQ ID NO: 14

SEQ ID NO: 17 - protein, 450 aa, synthetic construct
EVQLVESGGGLVQPGGSLRLSCAASGFNIKDTYIHWVRQAPGKGLEWVARIYPTNGYTRYADSVKGRFTISADTSKNTAYLQMNSLRAEDTAVYYCSRWGGDGFYAMDYWGQGTLVTVSSASTKGPSVFPLAPSSKSTSGGTAALGCLVKDYFPEPVTVSWNSGALTSGVHTFPAVLQSSGLYSLSSVVTVPSSSLGTQTYICNVNHKPSNTKVDKKVEPKSCDKTHTCPPCPAPELLGGPSVFLFPPKPKDTLMISRTPEVTCVVVDVSHEDPEVKFNWYVDGVEVHNAKTKPREEQYNSTYRVVSVLTVLHQDWLNGKEYKCKVSNKALPAPIEKTISKAKGQPREPQVYTLPPSREEMTKNQVSLTCLVKGFYPCDIAVEWESNGQPENNYKTTPPVLDSDGSFFLYSKLTVDKSRWQQGNVFSCSVMHEALHNHYTQKSLSLSPGK

SEQ ID NO: 18 - protein, 214 aa, synthetic construct
DIQMTQSPSSLSASVGDRVTITCRASQDVNTAVAWYQQKPGKAPKLLIYSASFLYSGVPSRFSGSRSGTDFTLTISSLQPEDFATYYCQQHYTTPPTFGQGTKVEIKRTCAAPSVFIFPPSDEQLKSGTASVVCLLNNFYPREAKVQWKVDNALQSGNSQESVTEQDSKDSTYSLSSTLTLSKADYEKHKVYACEVTHQGLSXPVTKSFNRGEC

SEQ ID NO: 19 - protein, 451 aa, synthetic construct
QVQLQQSGSELKKPGASVKVSCKASGYTFTNYGMNWVKQAPGQGLKWMGWINTYTGEPTYTDDFKGRFAFSLDTSVSTAYLQISSLKADDTAVYFCARGGFGSSYWYFDVWGQGSLVTVSSASTKGPSVFPLAPSSKSTSGGTAALGCLVKDYFPEPVTVSWNSGALTSGVHTFPAVLQSSGLYSLSSVVTVPSSSLGTQTYICNVNHKPSNTKVDKRVEPKSCDKTHTCPPCPAPELLGGPSVFLFPPKPKDTLMISRTPEVTCVVVDVSHEDPEVKFNWYVDGVEVHNAKTKPREEQYNSTYRVVSVLTVLHQDWLNGKEYKCKVSNKALPAPIEKTISKAKGQPREPQVYTLPPSREEMTKNQVSLTCLVKGFYPSDIAVEWESNGQPENNYKTTPPVLDSDGSFFLYSKLTVDKSRWQQGNVFSCSVMHEALHNHYTQKSLSLSPGK

SEQ ID NO: 20 - protein, 214 aa, synthetic construct
DIQLTQSPSSLSASVGDRVSITCKASQDVSIAVAWYQQKPGKAPKLLIYSASYRYTGVPDRFSGSGSGTDFTLTISSLQPEDFAVYYCQQHYITPLTFGAGTKVEIKRTVAAPSVFIFPPSDEQLKSGTASVVCLLNNFYPREAKVQWKVDNALQSGNSQESVTEQDSKDSTYSLSSTLTLSKADYEKHKVYACEVTHQGLSSPVTKSFNRGEC

SEQ ID NO: 21 - protein, 451 aa, synthetic construct
QVQLQQSGSELKKPGASVKVSCKASGYTFTNYGMNWVKQAPGQGLKWMGWINTYTGEPTYTDDFKGRFAFSLDTSVSTAYLQISSLKADDTAVYFCARGGFGSSYWYFDVWGQGSLVTVSSASTKGPSVFPLAPSSKSTSGGTAALGCLVKDYFPEPVTVSWNSGALTSGVHTFPAVLQSSGLYSLSSVVTVPSSSLGTQTYICNVNHKPSNTKVDKKVEPKSCDKTHTCPPCPAPELLGGPSVFLFPPKPKDTLMISRTPEVTCVVVDVSHEDPEVKFNWYVDGVEVHNAKTKPREEQYNSTYRVVSVLTVLHQDWLNGKEYKCKVSNKALPAPIEKTISKAKGQPREPQVYTLPPSREEMTKNQVSLTCLVKGFYPCDIAVEWESNGQPENNYKTTPPVLDSDGSFFLYSKLTVDKSRWQQGNVFSCSVMHEALHNHYTQKSLSLSPGK

SEQ ID NO: 22 - protein, 214 aa, synthetic construct
DIQLTQSPSSLSASVGDRVSITCKASQDVSIAVAWYQQKPGKAPKLLIYSASYRYTGVPDRFSGSGSGTDFTLTISSLQPEDFAVYYCQQHYITPLTFGAGTKVEIKRTCAAPSVFIFPPSDEQLKSGTASVVCLLNNFYPREAKVQWKVDNALQSGNSQESVTEQDSKDSTYSLSSTLTLSKADYEKHKVYACEVTHQGLSSPVTKSFNRGEC

SEQ ID NO: 23 - protein, 449 aa, synthetic construct
EVQLVESGGGVVQPGRSLRLSCSASGFTFSGYGLSWVRQAPGKGLEWVAMISSGGSYTYYADSVKGRFAISRDNAKNTLFLQMDSLRPEDTGVYFCARHGDDPAWFAYWGQGTPVTVSSASTKGPSVFPLAPSSKSTSGGTAALGCLVKDYFPCPVTVSWNSGALTSGVHTFPAVLQSSGLYSLSSVVTVPSSSLGTQTYICNVNHKPSNTKVDKKVEPKSCDKTHTCPPCPAPELLGGPSVFLFPPKPKDTLMISRTPEVTCVVVDVSHEDPEVKFNWYVDGVEVHNAKTKPREEQYNSTYRVVSVLTVLHQDWLNGKEYKCKVSNKALPAPIEKTISKAKGQPREPQVYTLPPSREEMTKNQVSLTCLVKGFYPCDIAVEWESNGQPENNYKTTPPVLDSDGSFFLYSKLTVDKSRWQQGNVFSCSVMHEALHNHYTQKSLSLSPGK

SEQ ID NO: 24 - protein, 217 aa, synthetic construct
DIQLTQSPSSLSASVGDRVTITCSVSSSISSNNLHWYQQKPGKAPKPWIYGTSNLASGVPSRFSGSGSGTDYTFTISSLQPEDIATYYCQQWSSYPYMYTFGQGTKVEIKRTVAAPSVFIFPPSDEQLKSGTASVVCLLNNFYPREAKVQWKVDNALQSGNSQESVTEQDSKDSTYSLSSTLTLSKADYEKHKVYACEVTHQGLSSPVTKSFNRGEC

SEQ ID NO: 25 - protein, 458 aa, synthetic construct
QVQLVESGGGVVRPGRSLRLSCAASGFAFSDYSINWVRQAPGKGLEWVAIISYDGRITYYRDSVKGRFTISRDDSKNTLYLQMNSLRTEDTAVYYCARQYYDFWSGSSVGRNYDGMDVWGLGTTVTVSSASTKGPSVFPLAPSSKSTSGGTAALGCLVKDYFPCPVTVSWNSGALTSGVHTFPAVLQSSGLYSLSSVVTVPSSSLGTQTYICNVNHKPSNTKVDKKVEPKSCDKTHTCPPCPAPELLGGPSVFLFPPKPKDTLMISRTPEVTCVVVDVSHEDPEVKFNWYVDGVEVHNAKTKPREEQYNSTYRVVSVLTVLHQDWLNGKEYKCKVSNKALPAPIEKTISKAKGQPREPQVYTLPPSREEMTKNQVSLTCLVKGFYPCDIAVEWESNGQPENNYKTTPPVLDSDGSFFLYSKLTVDKSRWQQGNVFSCSVMHEALHNHYTQKSLSLSPG

SEQ ID NO: 26 - protein, 219 aa, synthetic construct
DIVMTQSPLSLSVTPGEPASISCRSSQSLLHRSGNNYLDWYLQKPGHSPQLLIYVGSNRASGVPDRFSGSGSGTEYTLKISRVEAEDVGVYYCMQALQTPRTFGQGTKLEIKRTVAAPSVFIFPPSDEQLKSGTASVVCLLNNFYPREAKVQWKVDNALQSGNSQESVTEQDSKDSTYSLSSTLTLSKADYEKHKVYACEVTHQGLSSPVTKSFNRGEC

SEQ ID NO: 27 - DNA, 20 bp, synthetic construct
  source 1..20: mol_type = other DNA
aactccaccagcagacagtg

SEQ ID NO: 28 - DNA, 20 bp, synthetic construct
  source 1..20: mol_type = other DNA
ggtacctttgcaccctccag

SEQ ID NO: 29 - DNA, 26 bp, synthetic construct
  source 1..26: mol_type = other DNA
ggaggcttaattacacatgttctctg

SEQ ID NO: 30 - DNA, 24 bp, synthetic construct
  source 1..24: mol_type = other DNA
aagtgcatcatcgttgttcataca

SEQ ID NO: 31 - DNA, 18 bp, synthetic construct
  source 1..18: mol_type = other DNA
gtctgagtgggactcaag

SEQ ID NO: 32 - DNA, 18 bp, synthetic construct
  source 1..18: mol_type = other DNA
gcagggatgatttcaagc

SEQ ID NO: 33 - DNA, 20 bp, synthetic construct
  source 1..20: mol_type = other DNA
cccacgtcaaggagtatttc

SEQ ID NO: 34 - DNA, 20 bp, synthetic construct
  source 1..20: mol_type = other DNA
accctctatcctagctcatc

SEQ ID NO: 35 - DNA, 20 bp, synthetic construct
  source 1..20: mol_type = other DNA
ctgctgctttgcctacattg

SEQ ID NO: 36 - DNA, 20 bp, synthetic construct
  source 1..20: mol_type = other DNA
tcccgaacccatttcttctc

SEQ ID NO: 37 - DNA, 20 bp, synthetic construct
  source 1..20: mol_type = other DNA
gaagggtgagaagagatgtc

SEQ ID NO: 38 - DNA, 19 bp, synthetic construct
  source 1..19: mol_type = other DNA
tagggaagtgatgggagag